European Patent Specification EP 4 034 238 B1, published September 24, 2025. Title: ANTIBODIES FOR THE DIAGNOSIS AND/OR TREATMENT OF ATHEROSCLEROSIS. Applicant: Centro Nacional de Investigaciones Cardiovasculares Carlos III (F.S.P.) German Cancer Research Center, DKFZ. The sequence listing filed with the application follows.

SEQUENCE LISTING (146 sequences)

SEQ ID NO: 1 - protein, 8 aa, Artificial sequence
  Artificial sequence
GFTFSSYG

SEQ ID NO: 2 - protein, 8 aa, Artificial sequence
  Artificial sequence
ISSGGSYT

SEQ ID NO: 3 - protein, 15 aa, Artificial sequence
  Artificial sequence
ARPHVVTTPGWYFDV

SEQ ID NO: 4 - protein, 6 aa, Artificial sequence
  Artificial sequence
QSISDY

SEQ ID NO: 5 - protein, 3 aa, Artificial sequence
  Artificial sequence
YAS

SEQ ID NO: 6 - protein, 9 aa, Artificial sequence
  Artificial sequence
QNGHSFPLT

SEQ ID NO: 7 - protein, 8 aa, Artificial sequence
  Artificial sequence
GFTFSSYA

SEQ ID NO: 8 - protein, 8 aa, Artificial sequence
  Artificial sequence
ISDGGSYT

SEQ ID NO: 9 - protein, 13 aa, Artificial sequence
  Artificial sequence
ARDWVVSYWYFDV

SEQ ID NO: 10 - protein, 6 aa, Artificial sequence
  Artificial sequence
QSISDY

SEQ ID NO: 11 - protein, 3 aa, Artificial sequence
  Artificial sequence
YAS

SEQ ID NO: 12 - protein, 9 aa, Artificial sequence
  Artificial sequence
QNGHSFPLT

SEQ ID NO: 13 - protein, 8 aa, Artificial sequence
  Artificial sequence
GYTFTEYT

SEQ ID NO: 14 - protein, 8 aa, Artificial sequence
  Artificial sequence
FYPGSGSI

SEQ ID NO: 15 - protein, 12 aa, Artificial sequence
  Artificial sequence
ARHEVSYWYFDV

SEQ ID NO: 16 - protein, 6 aa, Artificial sequence
  Artificial sequence
QSISDY

SEQ ID NO: 17 - protein, 3 aa, Artificial sequence
  Artificial sequence
YAS

SEQ ID NO: 18 - protein, 9 aa, Artificial sequence
  Artificial sequence
QNGHSFPLT

SEQ ID NO: 19 - protein, 8 aa, Artificial sequence
  Artificial sequence
GFTFSSNG

SEQ ID NO: 20 - protein, 8 aa, Artificial sequence
  Artificial sequence
ISSGGSYT

SEQ ID NO: 21 - protein, 15 aa, Artificial sequence
  Artificial sequence
VRPPPMVTTYWYLDV

SEQ ID NO: 22 - protein, 6 aa, Artificial sequence
  Artificial sequence
QSISDY

SEQ ID NO: 23 - protein, 3 aa, Artificial sequence
  Artificial sequence
YAS

SEQ ID NO: 24 - protein, 9 aa, Artificial sequence
  Artificial sequence
QNGHSFPLT

SEQ ID NO: 25 - protein, 8 aa, Artificial sequence
  Artificial sequence
GYTFTSYW

SEQ ID NO: 26 - protein, 8 aa, Artificial sequence
  Artificial sequence
IYPSDSET

SEQ ID NO: 27 - protein, 15 aa, Artificial sequence
  Artificial sequence
ARGGYTTVVPRAMDY

SEQ ID NO: 28 - protein, 12 aa, Artificial sequence
  Artificial sequence
QSVLYSSNQKNY

SEQ ID NO: 29 - protein, 3 aa, Artificial sequence
  Artificial sequence
WAS

SEQ ID NO: 30 - protein, 8 aa, Artificial sequence
  Artificial sequence
HQYLSSLT

SEQ ID NO: 31 - protein, 8 aa, Artificial sequence
  Artificial sequence
GYTFTDYN

SEQ ID NO: 32 - protein, 8 aa, Artificial sequence
  Artificial sequence
INPNNGGT

SEQ ID NO: 33 - protein, 12 aa, Artificial sequence
  Artificial sequence
ARTVYYGNYVDY

SEQ ID NO: 34 - protein, 6 aa, Artificial sequence
  Artificial sequence
QDISNY

SEQ ID NO: 35 - protein, 3 aa, Artificial sequence
  Artificial sequence
YTS

SEQ ID NO: 36 - protein, 9 aa, Artificial sequence
  Artificial sequence
QQGNTLPLT

SEQ ID NO: 37 - protein, 8 aa, Artificial sequence
  Artificial sequence
GFTFNTYA

SEQ ID NO: 38 - protein, 10 aa, Artificial sequence
  Artificial sequence
IRSKSSNYAT

SEQ ID NO: 39 - protein, 13 aa, Artificial sequence
  Artificial sequence
VKAYGSSYWYFDV

SEQ ID NO: 40 - protein, 6 aa, Artificial sequence
  Artificial sequence
QSISDY

SEQ ID NO: 41 - protein, 3 aa, Artificial sequence
  Artificial sequence
YAS

SEQ ID NO: 42 - protein, 9 aa, Artificial sequence
  Artificial sequence
QNGHSFPLT

SEQ ID NO: 43 - protein, 8 aa, Artificial sequence
  Artificial sequence
GYTFTSYW

SEQ ID NO: 44 - protein, 8 aa, Artificial sequence
  Artificial sequence
IYPSDSET

SEQ ID NO: 45 - protein, 15 aa, Artificial sequence
  Artificial sequence
ARGGYTTVVPRAMDY

SEQ ID NO: 46 - protein, 12 aa, Artificial sequence
  Artificial sequence
QSVLYSSNQKNY

SEQ ID NO: 47 - protein, 3 aa, Artificial sequence
  Artificial sequence
WAS

SEQ ID NO: 48 - protein, 8 aa, Artificial sequence
  Artificial sequence
HQYLSSWT

SEQ ID NO: 49 - protein, 8 aa, Artificial sequence
  Artificial sequence
GYTFTEYT

SEQ ID NO: 50 - protein, 8 aa, Artificial sequence
  Artificial sequence
FYPGNNII

SEQ ID NO: 51 - protein, 12 aa, Artificial sequence
  Artificial sequence
ARHEYSNWYFDV

SEQ ID NO: 52 - protein, 6 aa, Artificial sequence
  Artificial sequence
QSISDY

SEQ ID NO: 53 - protein, 3 aa, Artificial sequence
  Artificial sequence
YAS

SEQ ID NO: 54 - protein, 9 aa, Artificial sequence
  Artificial sequence
QNGHSFPLT

SEQ ID NO: 55 - protein, 8 aa, Artificial sequence
  Artificial sequence
GYTFTEYT

SEQ ID NO: 56 - protein, 8 aa, Artificial sequence
  Artificial sequence
FYPGGVII

SEQ ID NO: 57 - protein, 12 aa, Artificial sequence
  Artificial sequence
ARHEYSNWYFDV

SEQ ID NO: 58 - protein, 6 aa, Artificial sequence
  Artificial sequence
QSISDY

SEQ ID NO: 59 - protein, 3 aa, Artificial sequence
  Artificial sequence
YAS

SEQ ID NO: 60 - protein, 9 aa, Artificial sequence
  Artificial sequence
QNGHSFPLT

SEQ ID NO: 61 - protein, 8 aa, Artificial sequence
  Artificial sequence
GFTFSSYG

SEQ ID NO: 62 - protein, 8 aa, Artificial sequence
  Artificial sequence
ISSGGSYT

SEQ ID NO: 63 - protein, 15 aa, Artificial sequence
  Artificial sequence
ARPPTLVTTYWYFDV

SEQ ID NO: 64 - protein, 6 aa, Artificial sequence
  Artificial sequence
QSISDY

SEQ ID NO: 65 - protein, 3 aa, Artificial sequence
  Artificial sequence
YAS

SEQ ID NO: 66 - protein, 9 aa, Artificial sequence
  Artificial sequence
QNGHSFPLT

SEQ ID NO: 67 - protein, 8 aa, Artificial sequence
  Artificial sequence
GFTFSSYA

SEQ ID NO: 68 - protein, 8 aa, Artificial sequence
  Artificial sequence
ISDGGSYT

SEQ ID NO: 69 - protein, 14 aa, Artificial sequence
  Artificial sequence
ARGRYGSSYWYFDV

SEQ ID NO: 70 - protein, 6 aa, Artificial sequence
  Artificial sequence
QSISDY

SEQ ID NO: 71 - protein, 3 aa, Artificial sequence
  Artificial sequence
YAS

SEQ ID NO: 72 - protein, 9 aa, Artificial sequence
  Artificial sequence
QNGHSFPLT

SEQ ID NO: 73 - protein, 8 aa, Artificial sequence
  Artificial sequence
GFSLTSYA

SEQ ID NO: 74 - protein, 7 aa, Artificial sequence
  Artificial sequence
IWTGGGT

SEQ ID NO: 75 - protein, 14 aa, Artificial sequence
  Artificial sequence
ASHYYGSSSWYFDV

SEQ ID NO: 76 - protein, 6 aa, Artificial sequence
  Artificial sequence
QSISDY

SEQ ID NO: 77 - protein, 3 aa, Artificial sequence
  Artificial sequence
YAS

SEQ ID NO: 78 - protein, 9 aa, Artificial sequence
  Artificial sequence
QNGHSFPLT

SEQ ID NO: 79 - protein, 8 aa, Artificial sequence
  Artificial sequence
GFTFSSYG

SEQ ID NO: 80 - protein, 8 aa, Artificial sequence
  Artificial sequence
ISSGGSYT

SEQ ID NO: 81 - protein, 16 aa, Artificial sequence
  Artificial sequence
ARQDYYGSSYGWYFDV

SEQ ID NO: 82 - protein, 6 aa, Artificial sequence
  Artificial sequence
QSISDY

SEQ ID NO: 83 - protein, 3 aa, Artificial sequence
  Artificial sequence
YAS

SEQ ID NO: 84 - protein, 8 aa, Artificial sequence
  Artificial sequence
QNGHSFPT

SEQ ID NO: 85 - protein, 8 aa, Artificial sequence
  Artificial sequence
GFTFSSYG

SEQ ID NO: 86 - protein, 8 aa, Artificial sequence
  Artificial sequence
ISSGGSYT

SEQ ID NO: 87 - protein, 16 aa, Artificial sequence
  Artificial sequence
ARHDYYGSSYGWYFDV

SEQ ID NO: 88 - protein, 6 aa, Artificial sequence
  Artificial sequence
QSISDY

SEQ ID NO: 89 - protein, 3 aa, Artificial sequence
  Artificial sequence
YAS

SEQ ID NO: 90 - protein, 9 aa, Artificial sequence
  Artificial sequence
QNGHSFPYT

SEQ ID NO: 91 - protein, 8 aa, Artificial sequence
  Artificial sequence
GYTFTDYY

SEQ ID NO: 92 - protein, 8 aa, Artificial sequence
  Artificial sequence
IFPGSGST

SEQ ID NO: 93 - protein, 15 aa, Artificial sequence
  Artificial sequence
ARWRYYGSSPYYFDY

SEQ ID NO: 94 - protein, 6 aa, Artificial sequence
  Artificial sequence
QSISDY

SEQ ID NO: 95 - protein, 3 aa, Artificial sequence
  Artificial sequence
YAS

SEQ ID NO: 96 - protein, 9 aa, Artificial sequence
  Artificial sequence
QNGHSFPLT

SEQ ID NO: 97 - protein, 8 aa, Artificial sequence
  Artificial sequence
GYTFTSYG

SEQ ID NO: 98 - protein, 8 aa, Artificial sequence
  Artificial sequence
IYPRSGNT

SEQ ID NO: 99 - protein, 14 aa, Artificial sequence
  Artificial sequence
ARLHDGYSTWYFDV

SEQ ID NO: 100 - protein, 6 aa, Artificial sequence
  Artificial sequence
QSIGTS

SEQ ID NO: 101 - protein, 3 aa, Artificial sequence
  Artificial sequence
YAS

SEQ ID NO: 102 - protein, 9 aa, Artificial sequence
  Artificial sequence
QQSNSWPFT

SEQ ID NO: 103 - protein, 8 aa, Artificial sequence
  Artificial sequence
GFTFSSYA

SEQ ID NO: 104 - protein, 8 aa, Artificial sequence
  Artificial sequence
ISDGGTYT

SEQ ID NO: 105 - protein, 14 aa, Artificial sequence
  Artificial sequence
GRDGLTGTVWYFDV

SEQ ID NO: 106 - protein, 6 aa, Artificial sequence
  Artificial sequence
QSISDY

SEQ ID NO: 107 - protein, 3 aa, Artificial sequence
  Artificial sequence
YAS

SEQ ID NO: 108 - protein, 9 aa, Artificial sequence
  Artificial sequence
QHGHSFPLT

SEQ ID NO: 109 - protein, 122 aa, Artificial sequence
  Artificial sequence
EVQLVESGGDLVKPGGSLKLSCAASGFTFSSYGMSWVRQTPDKRLEWVATISSGGSYTYYPDSVKGRFTISRDNAKNTLYLQMSSLKSEDTAMYYCARPHVVTTPGWYFDVWGTGTTVTVSS

SEQ ID NO: 110 - protein, 107 aa, Artificial sequence
  Artificial sequence
DIVMTQSPATLSVTPGDRVSLSCRASQSISDYLHWYQQKSHESPRLLIKYASQSISGIPSRFSGSGSGSDFTLSINSVEPEDVGVYYCQNGHSFPLTFGAGTKLELK

SEQ ID NO: 111 - protein, 120 aa, Artificial sequence
  Artificial sequence
EVQLVESGGGLVKPGGSLKLSCAASGFTFSSYAMSWVRQTPEKRLEWVATISDGGSYTYYPDNVKGRFTISRDNAKNNLYLQMSHLKSEDTAMYYCARDWVVSYWYFDVWGTGTTVTVSS

SEQ ID NO: 112 - protein, 107 aa, Artificial sequence; identical to SEQ ID NO: 110
  Artificial sequence

SEQ ID NO: 113 - protein, 119 aa, Artificial sequence
  Artificial sequence
QVQLQQSGAELVKPGASVKLSCKASGYTFTEYTIHWVKQRSGQGLEWIGWFYPGSGSIKYNEKFKDKATLTADKSSSTVYMELSRLTSEDSAVYFCARHEVSYWYFDVWGTGTTVTVSS

SEQ ID NO: 114 - protein, 107 aa, Artificial sequence; identical to SEQ ID NO: 110
  Artificial sequence

SEQ ID NO: 115 - protein, 122 aa, Artificial sequence
  Artificial sequence
EVQLVESGGDLVRPGGSLKLSCAASGFTFSSNGMSWVRQTPDKRLEWVATISSGGSYTYYPDSVKGRFTISRDNAKNTLYLQMSSLKSEDTAMYYCVRPPPMVTTYWYLDVWGTGTTVTVSS

SEQ ID NO: 116 - protein, 107 aa, Artificial sequence; identical to SEQ ID NO: 110
  Artificial sequence

SEQ ID NO: 117 - protein, 122 aa, Artificial sequence
  Artificial sequence
QVQLQQPGAELVRPGSSVKLSCKASGYTFTSYWMDWVKQRPGQGLEWIGNIYPSDSETHYNQKFKDKATLTVDKSSSTAYMQLSSLTSEDSAVYYCARGGYTTVVPRAMDYWGQGTSVTVSS

SEQ ID NO: 118 - protein, 112 aa, Artificial sequence
  Artificial sequence
NIMMTQSPSSLAVSAGEKVTMSCKSSQSVLYSSNQKNYLAWYQQKPGQSPKLLIYWASTRESGVPDRFTGSGSGTDFTLTISSVQAEDLAVYYCHQYLSSLTFGAGTKLELK

SEQ ID NO: 119 - protein, 119 aa, Artificial sequence
  Artificial sequence
EVQLQQSGPELVKPGASVKMSCKASGYTFTDYNMHWVKQSHGKSLEWIGYINPNNGGTSYNQKFKGKATLTVNKSSSTAYMELRSLTSEDSAVYYCARTVYYGNYVDYWGQGTTLTVSS

SEQ ID NO: 120 - protein, 107 aa, Artificial sequence
  Artificial sequence
DIQMTQTTSSLSASLGDRVTISCRASQDISNYLNWYQQKPDGTVKLLIYYTSRLHSGVPSRFSGSGSGTDYSLTISNLEQEDIATYFCQQGNTLPLTFGAGTKLELK

SEQ ID NO: 121 - protein, 122 aa, Artificial sequence
  Artificial sequence
EVQLVESGGGLVQPKGSLKLSCAASGFTFNTYAMHWVRQAPGKGLEWVARIRSKSSNYATYYADSVKDRFTISRDDSQSMLYLQMNNLKTEDTAMYYCVKAYGSSYWYFDVWGTGTTVTVSS

SEQ ID NO: 122 - protein, 107 aa, Artificial sequence; identical to SEQ ID NO: 110
  Artificial sequence

SEQ ID NO: 123 - protein, 122 aa, Artificial sequence; identical to SEQ ID NO: 117
  Artificial sequence

SEQ ID NO: 124 - protein, 112 aa, Artificial sequence
  Artificial sequence
NIMMTQSPSSLAVSAGEKVTMSCKSSQSVLYSSNQKNYLAWYQQKPGQSPKLLIYWASTRESGVPDRFTGSGSGTDFTLTISSVQAEDLAVYYCHQYLSSWTFGGGTKLEIK

SEQ ID NO: 125 - protein, 119 aa, Artificial sequence
  Artificial sequence
QVQLQQSGAELVKPGASVKLSCKASGYTFTEYTIHWVKQRSGQGLEWIGWFYPGNNIIKYNEKFKDKATLTADKSSSTVYMELSRLTSEDSAVYFCARHEYSNWYFDVWGTGTTVTVSS

SEQ ID NO: 126 - protein, 107 aa, Artificial sequence; identical to SEQ ID NO: 110
  Artificial sequence

SEQ ID NO: 127 - protein, 119 aa, Artificial sequence
  Artificial sequence
QVQLQQSGAELVKPGASVKLSCKASGYTFTEYTIHWVKQRSGQGLEWIGWFYPGGVIIKYNEKFKDKATLTADKSSSTVYMELSRLTSEDSAVYFCARHEYSNWYFDVWGTGTTVTVSS

SEQ ID NO: 128 - protein, 107 aa, Artificial sequence; identical to SEQ ID NO: 110
  Artificial sequence

SEQ ID NO: 129 - protein, 122 aa, Artificial sequence
  Artificial sequence
EVQLVESGGDLVKPGGSLKLSCAASGFTFSSYGMSWVRQTPDKRLEWVATISSGGSYTYYPDSVKGRFTISRDNAKNTLHLQMSSLKSEDTAMYYCARPPTLVTTYWYFDVWGTGTTVTVSS

SEQ ID NO: 130 - protein, 107 aa, Artificial sequence; identical to SEQ ID NO: 110
  Artificial sequence

SEQ ID NO: 131 - protein, 121 aa, Artificial sequence
  Artificial sequence
EVQLVESGGGLVKPGGSLKLSCAASGFTFSSYAMSWVRQTPEKRLEWVATISDGGSYTYYPDNVKGRFTISRDNAKNNLYLQMSHLKSEDTAMYYCARGRYGSSYWYFDVWGTGTTVTVSS

SEQ ID NO: 132 - protein, 107 aa, Artificial sequence
  Artificial sequence
DIVMTQSPATLSVTPGDKVSLSCRASQSISDYLHWYQQKSHESPRLLIKYASQSISGIPSRFSGSGSGSDFTLSINSVEPEDVGVYYCQNGHSFPLTFGAGTKLELK

SEQ ID NO: 133 - protein, 120 aa, Artificial sequence
  Artificial sequence
QVQLKESGPGLVAPSQSLSITCTVSGFSLTSYAISWVRQPPGKGLEWLGVIWTGGGTNYNSALKSRLSISKDNSKSQVFLKMNSLQTDDTARYYCASHYYGSSSWYFDVWGTGTTVTVSS

SEQ ID NO: 134 - protein, 107 aa, Artificial sequence; identical to SEQ ID NO: 110
  Artificial sequence

SEQ ID NO: 135 - protein, 123 aa, Artificial sequence
  Artificial sequence
EVQLVESGGDLVKPGGSLKLSCAASGFTFSSYGMSWVRQTPDKRLEWVATISSGGSYTYYPDSVKGRFTISRDNAKNTLYLQMSSLKSEDTAMYYCARQDYYGSSYGWYFDVWGTGTTVTVSS

SEQ ID NO: 136 - protein, 106 aa, Artificial sequence
  Artificial sequence
DIVMTQSPATLSVTPGDRVSLSCRASQSISDYLHWYQQKSHESPRLLIKYASQSISGIPSRFSGSGSGSDFTLSINSVEPEDVGVYYCQNGHSFPTFGGGTKLEIK

SEQ ID NO: 137 - protein, 123 aa, Artificial sequence
  Artificial sequence
EVQLVESGGDLVKPGGSLKLSCAASGFTFSSYGMSWVRQTPDKRLEWVATISSGGSYTYYPDSVKGRFTISRDNAKNTLYLQMSSLKSEDTAMYYCARHDYYGSSYGWYFDVWGTGTTVTVSS

SEQ ID NO: 138 - protein, 107 aa, Artificial sequence
  Artificial sequence
DIVMTQSPATLSVTPGDRVSLSCRASQSISDYLHWYQQKSHESPRLLIKYASQSISGIPSRFSGSGSGSDFTLSINSVEPEDVGVYYCQNGHSFPYTFGGETKLEIK

SEQ ID NO: 139 - protein, 122 aa, Artificial sequence
  Artificial sequence
QVQLQQSGPELVKPGASVKISCKASGYTFTDYYINWVKQRPGQGLEWIGWIFPGSGSTYYDYYINWVKQRPGQGLEWIGWIFPGSGSTYYSAVYFCARWRYYGSSPYYFDYWGQGTTLTVSS

SEQ ID NO: 140 - protein, 107 aa, Artificial sequence
  Artificial sequence
DIVMTQSPATLSVTPGDRASLSCRASQSISDYLHWYQQKSHESPRLLIKYASQSISGIPSRFSGSGSGSDFTLSINSVEPEDVGVYYCQNGHSFPLTFGAGTKLELK

SEQ ID NO: 141 - protein, 121 aa, Artificial sequence
  Artificial sequence
QVQLQQSGAELARPGASVKLSCKASGYTFTSYGISWVKQRTGQGLEWIGEIYPRSGNTYYNEKFKGKATLTADKSSSTAYMELRSLTSEDSAVYFCARLHDGYSTWYFDVWGTGTTVTVSS

SEQ ID NO: 142 - protein, 107 aa, Artificial sequence
  Artificial sequence
DILLTQSPAILSVSPGERVSFSCRASQSIGTSIHWYQQRTNGSPRLLIKYASESISGIPSRFSGSGSGTDFTLSINSVESEDIADYYCQQSNSWPFTFGSGTKLEIK

SEQ ID NO: 143 - protein, 121 aa, Artificial sequence
  Artificial sequence
EVQLVESGGGLVKPGGSLKLSCAASGFTFSSYAMSWVRQTPEKRLEWVATISDGGTYTYYLDNVKGRFTISRDNAKNNLYLQMSHLKSEDTAMYYCGRDGLTGTVWYFDVWGTGTTVTVSS

SEQ ID NO: 144 - protein, 107 aa, Artificial sequence
  Artificial sequence
DIVMTQSPATLSVTPGDRVSLSCRASQSISDYLHWYQQKSHESPRLLIKYASQSISGIPSRFSGSGSGSDFTLSINCVEPEDVGVYYCQHGHSFPLTFGAGTKLELK

SEQ ID NO: 145 - DNA, 25 bp, Artificial sequence
  Artificial sequence
cagaggggaagacatgttcaactat

SEQ ID NO: 146 - DNA, 26 bp, Artificial sequence
  Artificial sequence
cagtggctgacttccaattactaaac